European Patent Specification EP 3 689 139 B1, published January 1, 2025. Title: NON-HUMAN ANIMALS HAVING A DISRUPTION IN A C9ORF72 LOCUS. Applicant: Regeneron Pharmaceuticals, Inc. The sequence listing filed with the application follows.

SEQUENCE LISTING (9 sequences)

SEQ ID NO: 1 - DNA, 3198 bp, Mus musculus
gtgtccggggcggggcggtcccggggcggggcccggagcgggctgcggttgcggtccctgcgccggcggtgaaggcgcagcagcggcgagtggctattgcaagcgttcggataatgtgagacctggaatgcagtgagacctgggatgcagggatgtcgactatctgccccccaccatctcctgctgttgccaagacagagattgctttaagtggtgaatcacccttgttggcggctacctttgcttactgggataatattcttggtcctagagtaaggcatatttgggctccaaagacagaccaagtgcttctcagtgatggagaaataacttttcttgccaaccacactctaaatggagaaattcttcgaaatgcagagagtggggctatagatgtaaaattttttgtcttatctgaaaaaggggtaattattgtttcattaatcttcgacggaaactggaatggagatcggagcacttatggactatcaattatactgccgcagacagagctgagcttctacctcccacttcacagagtgtgtgttgacaggctaacacacattattcgaaaaggaagaatatggatgcataaggaaagacaagaaaatgtccagaaaattgtcttggaaggcacagagaggatggaagatcagggtcagagtatcattcccatgcttactggggaagtcattcctgtaatggagctgcttgcatctatgaaatcccacagtgttcctgaagacattgatatagctgatacagtgctcaatgatgatgacattggtgacagctgtcacgaaggctttcttctcaatgccatcagctcacacctgcagacctgtggctgttccgttgtagttggcagcagtgcagagaaagtaaataagatagtaagaacgctgtgcctttttctgacaccagcagagaggaaatgctccaggctgtgtgaagcagaatcgtcctttaagtacgaatcgggactctttgtgcaaggcttgctaaaggatgcaacaggcagttttgtcctacccttccggcaagttatgtatgccccgtaccccaccacgcacattgatgtggatgtcaacactgtcaagcagatgccaccgtgtcatgaacatatttataatcaacgcagatacatgaggtcagagctgacagccttctggagggcaacttcagaagaggacatggcgcaggacaccatcatctacacagatgagagcttcactcctgatttgaatattttccaagatgtcttacacagagacactctagtgaaagccttcctggatcaggtcttccatttgaagcctggcctgtctctcaggagtactttccttgcacagttcctcctcattcttcacagaaaagccttgacactaatcaagtacatcgaggatgatacgcagaaggggaaaaagccctttaagtctcttcggaacctgaagatagatcttgatttaacagcagagggcgatcttaacataataatggctctagctgagaaaattaagccaggcctacactctttcatctttgggagacctttctacactagtgtacaagaacgtgatgttctaatgaccttttgaccgtgtggtttgctgtgtctgtctcttcacagtcacacctgctgttacagtgtctcagcagtgtgtgggcacatccttcctcccgagtcctgctgcaggacagggtacactacacttgtcagtagaagtctgtacctgatgtcaggtgcatcgttacagtgaatgactcttcctagaatagatgtactcttttagggccttatgtttacaattatcctaagtactattgctgtcttttaaagatatgaatgatggaatatacacttgaccataactgctgattggttttttgttttgttttgtttgttttcttggaaacttatgattcctggtttacatgtaccacactgaaaccctcgttagctttacagataaagtgtgagttgacttcctgcccctctgtgttctgtggtatgtccgattacttctgccacagctaaacattagagcatttaaagtttgcagttcctcagaaaggaacttagtctgactacagattagttcttgagagaagacactgatagggcagagctgtaggtgaaatcagttgttagcccttcctttatagacgtagtccttcagattcggtctgtacagaaatgccgaggggtcatgcatgggccctgagtatcgtgacctgtgacaagttttttgttggtttattgtagttctgtcaaagaaagtggcatttgtttttataattgttgccaacttttaaggttaattttcattatttttgagccgaattaaaatgcgcacctcctgtgcctttcccaatcttggaaaatataatttcttggcagagggtcagatttcagggcccagtcactttcatctgaccaccctttgcacggctgccgtgtgcctggcttagattagaagtccttgttaagtatgtcagagtacattcgctgataagatctttgaagagcagggaagcgtcttgcctctttcctttggtttctgcctgtactctggtgtttcccgtgtcacctgcatcataggaacagcagagaaatctgacccagtgctatttttctaggtgctactatggcaaactcaagtggtctgtttctgttcctgtaacgttcgactatctcgctagctgtgaagtactgattagtggagttctgtgcaacagcagtgtaggagtatacacaaacacaaatatgtgtttctatttaaaactgtggacttagcataaaaagggagaatatatttattttttacaaaagggataaaaatgggccccgttcctcacccaccagatttagcgagaaaaagctttctattctgaaaggtcacggtggctttggcattacaaatcagaacaacacacactgaccatgatggcttgtgaactaactgcaaggcactccgtcatggtaagcgagtaggtcccacctcctagtgtgccgctcattgctttacacagtagaatcttatttgagtgctaattgttgtctttgctgctttactgtgttgttatagaaaatgtaagctgtacagtgaataagttattgaagcatgtgtaaacactgttatatatcttttctcctagatggggaattttgaataaaatacctttgaaattctgtgt

SEQ ID NO: 2 - protein, 481 aa, 2 481 PRT Mus musculus
MSTICPPPSPAVAKTEIALSGESPLLAATFAYWDNILGPRVRHIWAPKTDQVLLSDGEITFLANHTLNGEILRNAESGAIDVKFFVLSEKGVIIVSLIFDGNWNGDRSTYGLSIILPQTELSFYLPLHRVCVDRLTHIIRKGRIWMHKERQENVQKIVLEGTERMEDQGQSIIPMLTGEVIPVMELLASMKSHSVPEDIDIADTVLNDDDIGDSCHEGFLLNAISSHLQTCGCSVVVGSSAEKVNKIVRTLCLFLTPAERKCSRLCEAESSFKYESGLFVQGLLKDATGSFVLPFRQVMYAPYPTTHIDVDVNTVKQMPPCHEHIYNQRRYMRSELTAFWRATSEEDMAQDTIIYTDESFTPDLNIFQDVLHRDTLVKAFLDQVFHLKPGLSLRSTFLAQFLLILHRKALTLIKYIEDDTQKGKKPFKSLRNLKIDLDLTAEGDLNIIMALAEKIKPGLHSFIFGRPFYTSVQERDVLMTF

SEQ ID NO: 3 - DNA, 3435 bp, Rattus norvegicus
cgtttgtagtgtcagccatcccaattgcctgttccttctctgtgggagtggtgtctagacagtccaggcagggtatgctaggcaggtgcgttttggttgcctcagatcgcaacttgactccataacggtgaccaaagacaaaagaaggaaaccagattaaaaagaaccggacacagacccctgcagaatctggagcggccgtggttgggggcggggctacgacggggcggactcgggggcgtgggagggcggggccggggcggggcccggagccggctgcggttgcggtccctgcgccggcggtgaaggcgcagcggcggcgagtggctattgcaagcgtttggataatgtgagacctgggatgcagggatgtcgactatctgccccccaccatctcctgctgttgccaagacagagattgctttaagtggtgaatcacccttgttggcggctacctttgcttactgggataatattcttggtcctagagtaaggcacatttgggctccaaagacagaccaagtactcctcagtgatggagaaatcacttttcttgccaaccacactctgaatggagaaattcttcggaatgcggagagtggggcaatagatgtaaagttttttgtcttatctgaaaagggcgtcattattgtttcattaatcttcgacgggaactggaacggagatcggagcacttacggactatcaattatactgccgcagacggagctgagtttctacctcccactgcacagagtgtgtgttgacaggctaacgcacatcattcgaaaaggaaggatatggatgcacaaggaaagacaagaaaatgtccagaaaattgtcttggaaggcaccgagaggatggaagatcagggtcagagtatcatccctatgcttactggggaggtcatccctgtgatggagctgcttgcgtctatgagatcacacagtgttcctgaagacctcgatatagctgatacagtactcaatgatgatgacattggtgacagctgtcatgaaggctttcttctcaatgccatcagctcacatctgcagacctgcggctgttctgtggtggtaggcagcagtgcagagaaagtaaataagatagtaagaacactgtgcctttttctgacaccagcagagaggaagtgctccaggctgtgtgaagccgaatcgtcctttaaatacgaatctggactctttgtacaaggcttgctaaaggatgcgactggcagttttgtactacctttccggcaagttatgtatgccccttatcccaccacacacatcgatgtggatgtcaacactgtcaagcagatgccaccgtgtcatgaacatatttataatcaacgcagatacatgaggtcagagctgacagccttctggagggcaacttcagaagaggacatggctcaggacaccatcatctacacagatgagagcttcactcctgatttgaatattttccaagatgtcttacacagagacactctagtgaaagcctttctggatcaggtcttccatttgaagcctggcctgtctctcaggagtactttccttgcacagttcctcctcattcttcacagaaaagccttgacactaatcaagtacatagaggatgacacgcagaaggggaaaaagccctttaagtctcttcggaacctgaagatagatcttgatttaacagcagagggcgaccttaacataataatggctctagctgagaaaattaagccaggcctacactctttcatcttcgggagacctttctacactagtgtccaagaacgtgatgttctaatgactttttaaacatgtggtttgctccgtgtgtctcatgacagtcacacttgctgttacagtgtctcagcgctttggacacatccttcctccagggtcctgccgcaggacacgttacactacacttgtcagtagaggtctgtaccagatgtcaggtacatcgttgtagtgaatgtctcttttcctagactagatgtaccctcgtagggacttatgtttacaaccctcctaagtactagtgctgtcttgtaaggatacgaatgaagggatgtaaacttcaccacaactgctggttggttttgttgtttttgttttttgaaacttataattcatggtttacatgcatcacactgaaaccctagttagctttttacaggtaagctgtgagttgactgcctgtccctgtgttctctggcctgtacgatctgtggcgtgtaggatcacttttgcaacaactaaaaactaaagcactttgtttgcagttctacagaaagcaacttagtctgtctgcagattcgtttttgaaagaagacatgagaaagcggagttttaggtgaagtcagttgttggatcttcctttatagacttagtcctttagatgtggtctgtatagacatgcccaaccatcatgcatgggcactgaatatcgtgaactgtggtatgctttttgttggtttattgtacttctgtcaaagaaagtggcattggtttttataattgttgccaagttttaaggttaattttcattatttttgagccaaattaaaatgtgcacctcctgtgcctttcccaatcttggaaaatataatttcttggcagaaggtcagatttcagggcccagtcactttcgtctgacttccctttgcacagtccgccatgggcctggcttagaagttcttgtaaactatgccagagagtacattcgctgataaaatcttctttgcagagcaggagagcttcttgcctctttcctttcatttctgcctggactttggtgttctccacgttccctgcatcctaaggacagcaggagaactctgaccccagtgctatttctctaggtgctattgtggcaaactcaagcggtccgtctctgtccctgtaacgttcgtaccttgctggctgtgaagtactgactggtaaagctccgtgctacagcagtgtagggtatacacaaacacaagtaagtgttttatttaaaactgtggacttagcataaaaagggagactatatttattttttacaaaagggataaaaatggaaccctttcctcacccaccagatttagtcagaaaaaaacattctattctgaaaggtcacagtggttttgacatgacacatcagaacaacgcacactgtccatgatggcttatgaactccaagtcactccatcatggtaaatgggtagatccctccttctagtgtgccacaccattgcttcccacagtagaatcttatttaagtgctaagtgttgtctctgctggtttactctgttgttttagagaatgtaagttgtatagtgaataagttattgaagcatgtgtaaacactgttatacatcttttctcctagatggggaatttggaataaaatacctttaaaattcaaaaaaaaaaaaaaaaaaaaaaaa

SEQ ID NO: 4 - protein, 481 aa, Rattus norvegicus
MSTICPPPSPAVAKTEIALSGESPLLAATFAYWDNILGPRVRHIWAPKTDQVLLSDGEITFLANHTLNGEILRNAESGAIDVKFFVLSEKGVIIVSLIFDGNWNGDRSTYGLSIILPQTELSFYLPLHRVCVDRLTHIIRKGRIWMHKERQENVQKIVLEGTERMEDQGQSIIPMLTGEVIPVMELLASMRSHSVPEDLDIADTVLNDDDIGDSCHEGFLLNAISSHLQTCGCSVVVGSSAEKVNKIVRTLCLFLTPAERKCSRLCEAESSFKYESGLFVQGLLKDATGSFVLPFRQVMYAPYPTTHIDVDVNTVKQMPPCHEHIYNQRRYMRSELTAFWRATSEEDMAQDTIIYTDESFTPDLNIFQDVLHRDTLVKAFLDQVFHLKPGLSLRSTFLAQFLLILHRKALTLIKYIEDDTQKGKKPFKSLRNLKIDLDLTAEGDLNIIMALAEKIKPGLHSFIFGRPFYTSVQERDVLMTF

SEQ ID NO: 5 - DNA, 680 bp, Artificial Sequence
  Synthetic polynucleotide-prot promoter
ccagtagcagcacccacgtccaccttctgtctagtaatgtccaacacctccctcagtccaaacactgctctgcatccatgtggctcccatttatacctgaagcacttgatggggcctcaatgttttactagagcccacccccctgcaactctgagaccctctggatttgtctgtcagtgcctcactggggcgttggataatttcttaaaaggtcaagttccctcagcagcattctctgagcagtctgaagatgtgtgcttttcacagttcaaatccatgtggctgtttcacccacctgcctggccttgggttatctatcaggacctagcctagaagcaggtgtgtggcacttaacacctaagctgagtgactaactgaacactcaagtggatgccatctttgtcacttcttgactgtgacacaagcaactcctgatgccaaagccctgcccacccctctcatgcccatatttggacatggtacaggtcctcactggccatggtctgtgaggtcctggtcctctttgacttcataattcctaggggccactagtatctataagaggaagagggtgctggctcccaggccacagcccacaaaattccacctgctcacaggttggctggctcgacccaggtggtgtcccctgctctgagccagctcccggccaagccagcacc

SEQ ID NO: 6 - DNA, 1052 bp, Artificial Sequence
  Synthetic polynucleotide-Blimp1 promoter 1kb
tgccatcatcacaggatgtccttccttctccagaagacagactggggctgaaggaaaagccggccaggctcagaacgagccccactaattactgcctccaacagctttccactcactgcccccagcccaacatcccctttttaactgggaagcattcctactctccattgtacgcacacgctcggaagcctggctgtgggtttgggcatgagaggcagggacaacaaaaccagtatatatgattataactttttcctgtttccctatttccaaatggtcgaaaggaggaagttaggtctacctaagctgaatgtattcagttagcaggagaaatgaaatcctatacgtttaatactagaggagaaccgccttagaatatttatttcattggcaatgactccaggactacacagcgaaattgtattgcatgtgctgccaaaatactttagctctttccttcgaagtacgtcggatcctgtaattgagacaccgagtttaggtgactagggttttcttttgaggaggagtcccccaccccgccccgctctgccgcgacaggaagctagcgatccggaggacttagaatacaatcgtagtgtgggtaaacatggagggcaagcgcctgcaaagggaagtaagaagattcccagtccttgttgaaatccatttgcaaacagaggaagctgccgcgggtcgcagtcggtggggggaagccctgaaccccacgctgcacggctgggctggccaggtgcggccacgcccccatcgcggcggctggtaggagtgaatcagaccgtcagtattggtaaagaagtctgcggcagggcagggagggggaagagtagtcagtcgctcgctcactcgctcgctcgcacagacactgctgcagtgacactcggccctccagtgtcgcggagacgcaagagcagcgcgcagcacctgtccgcccggagcgagcccggcccgcggccgtagaaaaggagggaccgccgaggtgcgcgtcagtactgctcagcccggcagggacgcgggaggatgtggactgggtggac

SEQ ID NO: 7 - DNA, 2008 bp, Artificial Sequence
  Synthetic polynucleotide-Blimp1 promoter 2kb
gtggtgctgactcagcatcggttaataaaccctctgcaggaggctggatttcttttgtttaattatcacttggacctttctgagaactcttaagaattgttcattcgggtttttttgttttgttttggtttggtttttttgggttttttttttttttttttttttggtttttggagacagggtttctctgtatatagccctggcacaagagcaagctaacagcctgtttcttcttggtgctagcgccccctctggcagaaaatgaaataacaggtggacctacaacccccccccccccccccagtgtattctactcttgtccccggtataaatttgattgttccgaactacataaattgtagaaggattttttagatgcacatatcattttctgtgataccttccacacacccctcccccccaaaaaaatttttctgggaaagtttcttgaaaggaaaacagaagaacaagcctgtctttatgattgagttgggcttttgttttgctgtgtttcatttcttcctgtaaacaaatactcaaatgtccacttcattgtatgactaagttggtatcattaggttgggtctgggtgtgtgaatgtgggtgtggatctggatgtgggtgggtgtgtatgccccgtgtgtttagaatactagaaaagataccacatcgtaaacttttgggagagatgatttttaaaaatgggggtgggggtgaggggaacctgcgatgaggcaagcaagataaggggaagacttgagtttctgtgatctaaaaagtcgctgtgatgggatgctggctataaatgggcccttagcagcattgtttctgtgaattggaggatccctgctgaaggcaaaagaccattgaaggaagtaccgcatctggtttgttttgtaatgagaagcaggaatgcaaggtccacgctcttaataataaacaaacaggacattgtatgccatcatcacaggatgtccttccttctccagaagacagactggggctgaaggaaaagccggccaggctcagaacgagccccactaattactgcctccaacagctttccactcactgcccccagcccaacatcccctttttaactgggaagcattcctactctccattgtacgcacacgctcggaagcctggctgtgggtttgggcatgagaggcagggacaacaaaaccagtatatatgattataactttttcctgtttccctatttccaaatggtcgaaaggaggaagttaggtctacctaagctgaatgtattcagttagcaggagaaatgaaatcctatacgtttaatactagaggagaaccgccttagaatatttatttcattggcaatgactccaggactacacagcgaaattgtattgcatgtgctgccaaaatactttagctctttccttcgaagtacgtcggatcctgtaattgagacaccgagtttaggtgactagggttttcttttgaggaggagtcccccaccccgccccgctctgccgcgacaggaagctagcgatccggaggacttagaatacaatcgtagtgtgggtaaacatggagggcaagcgcctgcaaagggaagtaagaagattcccagtccttgttgaaatccatttgcaaacagaggaagctgccgcgggtcgcagtcggtggggggaagccctgaaccccacgctgcacggctgggctggccaggtgcggccacgcccccatcgcggcggctggtaggagtgaatcagaccgtcagtattggtaaagaagtctgcggcagggcagggagggggaagagtagtcagtcgctcgctcactcgctcgctcgcacagacactgctgcagtgacactcggccctccagtgtcgcggagacgcaagagcagcgcgcagcacctgtccgcccggagcgagcccggcccgcggccgtagaaaaggagggaccgccgaggtgcgcgtcagtactgctcagcccggcagggacgcgggaggatgtggactgggtggac

SEQ ID NO: 8 - DNA, 8388 bp, Artificial Sequence
  Polynucleotide sequence of a modified C9ORF72 locus from lacZ through the 3' loxP site
ggtaccgatttaaatgatccagtggtcctgcagaggagagattgggagaatcccggtgtgacacagctgaacagactagccgcccaccctccctttgcttcttggagaaacagtgaggaagctaggacagacagaccaagccagcaactcagatctttgaacggggagtggagatttgcctggtttccggcaccagaagcggtgccggaaagctggctggagtgcgatcttcctgaggccgatactgtcgtcgtcccctcaaactggcagatgcacggttacgatgcgcccatctacaccaacgtgacctatcccattacggtcaatccgccgtttgttcccacggagaatccgacgggttgttactcgctcacatttaatgttgatgaaagctggctacaggaaggccagacgcgaattatttttgatggcgttaactcggcgtttcatctgtggtgcaacgggcgctgggtcggttacggccaggacagtcgtttgccgtctgaatttgacctgagcgcatttttacgcgccggagaaaaccgcctcgcggtgatggtgctgcgctggagtgacggcagttatctggaagatcaggatatgtggcggatgagcggcattttccgtgacgtctcgttgctgcataaaccgactacacaaatcagcgatttccatgttgccactcgctttaatgatgatttcagccgcgctgtactggaggctgaagttcagatgtgcggcgagttgcgtgactacctacgggtaacagtttctttatggcagggtgaaacgcaggtcgccagcggcaccgcgcctttcggcggtgaaattatcgatgagcgtggtggttatgccgatcgcgtcacactacgtctgaacgtcgaaaacccgaaactgtggagcgccgaaatcccgaatctctatcgtgcggtggttgaactgcacaccgccgacggcacgctgattgaagcagaagcctgcgatgtcggtttccgcgaggtgcggattgaaaatggtctgctgctgctgaacggcaagccgttgctgattcgaggcgttaaccgtcacgagcatcatcctctgcatggtcaggtcatggatgagcagacgatggtgcaggatatcctgctgatgaagcagaacaactttaacgccgtgcgctgttcgcattatccgaaccatccgctgtggtacacgctgtgcgaccgctacggcctgtatgtggtggatgaagccaatattgaaacccacggcatggtgccaatgaatcgtctgaccgatgatccgcgctggctaccggcgatgagcgaacgcgtaacgcgaatggtgcagcgcgatcgtaatcacccgagtgtgatcatctggtcgctggggaatgaatcaggccacggcgctaatcacgacgcgctgtatcgctggatcaaatctgtcgatccttcccgcccggtgcagtatgaaggcggcggagccgacaccacggccaccgatattatttgcccgatgtacgcgcgcgtggatgaagaccagcccttcccggctgtgccgaaatggtccatcaaaaaatggctttcgctacctggagagacgcgcccgctgatcctttgcgaatacgcccacgcgatgggtaacagtcttggcggtttcgctaaatactggcaggcgtttcgtcagtatccccgtttacagggcggcttcgtctgggactgggtggatcagtcgctgattaaatatgatgaaaacggcaacccgtggtcggcttacggcggtgattttggcgatacgccgaacgatcgccagttctgtatgaacggtctggtctttgccgaccgcacgccgcatccagcgctgacggaagcaaaacaccagcagcagtttttccagttccgtttatccgggcaaaccatcgaagtgaccagcgaatacctgttccgtcatagcgataacgagctcctgcactggatggtggcgctggatggtaagccgctggcaagcggtgaagtgcctctggatgtcgctccacaaggtaaacagttgattgaactgcctgaactaccgcagccggagagcgccgggcaactctggctcacagtacgcgtagtgcaaccgaacgcgaccgcatggtcagaagccgggcacatcagcgcctggcagcagtggcgtctggcggaaaacctcagtgtgacgctccccgccgcgtcccacgccatcccgcatctgaccaccagcgaaatggatttttgcatcgagctgggtaataagcgttggcaatttaaccgccagtcaggctttctttcacagatgtggattggcgataaaaaacaactgctgacgccgctgcgcgatcagttcacccgtgcaccgctggataacgacattggcgtaagtgaagcgacccgcattgaccctaacgcctgggtcgaacgctggaaggcggcgggccattaccaggccgaagcagcgttgttgcagtgcacggcagatacacttgctgatgcggtgctgattacgaccgctcacgcgtggcagcatcaggggaaaaccttatttatcagccggaaaacctaccggattgatggtagtggtcaaatggcgattaccgttgatgttgaagtggcgagcgatacaccgcatccggcgcggattggcctgaactgccagctggcgcaggtagcagagcgggtaaactggctcggattagggccgcaagaaaactatcccgaccgccttactgccgcctgttttgaccgctgggatctgccattgtcagacatgtataccccgtacgtcttcccgagcgaaaacggtctgcgctgcgggacgcgcgaattgaattatggcccacaccagtggcgcggcgacttccagttcaacatcagccgctacagtcaacagcaactgatggaaaccagccatcgccatctgctgcacgcggaagaaggcacatggctgaatatcgacggtttccatatggggattggtggcgacgactcctggagcccgtcagtatcggcggaattccagctgagcgccggtcgctaccattaccagttggtctggtgtcaaaaataataataaccgggcaggggggatctaagctctagataagtaatgatcataatcagccatatcacatctgtagaggttttacttgctttaaaaaacctcccacacctccccctgaacctgaaacataaaatgaatgcaattgttgttgttaacttgtttattgcagcttataatggttacaaataaagcaatagcatcacaaatttcacaaataaagcatttttttcactgcattctagttgtggtttgtccaaactcatcaatgtatcttatcatgtctggatcccccggctagagtttaaacactagaactagtggatccccgggctcgataactataacggtcctaaggtagcgactcgagataacttcgtataatgtatgctatacgaagttatatgcatggcctccgcgccgggttttggcgcctcccgcgggcgcccccctcctcacggcgagcgctgccacgtcagacgaagggcgcagcgagcgtcctgatccttccgcccggacgctcaggacagcggcccgctgctcataagactcggccttagaaccccagtatcagcagaaggacattttaggacgggacttgggtgactctagggcactggttttctttccagagagcggaacaggcgaggaaaagtagtcccttctcggcgattctgcggagggatctccgtggggcggtgaacgccgatgattatataaggacgcgccgggtgtggcacagctagttccgtcgcagccgggatttgggtcgcggttcttgtttgtggatcgctgtgatcgtcacttggtgagtagcgggctgctgggctggccggggctttcgtggccgccgggccgctcggtgggacggaagcgtgtggagagaccgccaagggctgtagtctgggtccgcgagcaaggttgccctgaactgggggttggggggagcgcagcaaaatggcggctgttcccgagtcttgaatggaagacgcttgtgaggcgggctgtgaggtcgttgaaacaaggtggggggcatggtgggcggcaagaacccaaggtcttgaggccttcgctaatgcgggaaagctcttattcgggtgagatgggctggggcaccatctggggaccctgacgtgaagtttgtcactgactggagaactcggtttgtcgtctgttgcgggggcggcagttatggcggtgccgttgggcagtgcacccgtacctttgggagcgcgcgccctcgtcgtgtcgtgacgtcacccgttctgttggcttataatgcagggtggggccacctgccggtaggtgtgcggtaggcttttctccgtcgcaggacgcagggttcgggcctagggtaggctctcctgaatcgacaggcgccggacctctggtgaggggagggataagtgaggcgtcagtttctttggtcggttttatgtacctatcttcttaagtagctgaagctccggttttgaactatgcgctcggggttggcgagtgtgttttgtgaagttttttaggcaccttttgaaatgtaatcatttgggtcaatatgtaattttcagtgttagactagtaaattgtccgctaaattctggccgtttttggcttttttgttagacgtgttgacaattaatcatcggcatagtatatcggcatagtataatacgacaaggtgaggaactaaaccatgggatcggccattgaacaagatggattgcacgcaggttctccggccgcttgggtggagaggctattcggctatgactgggcacaacagacaatcggctgctctgatgccgccgtgttccggctgtcagcgcaggggcgcccggttctttttgtcaagaccgacctgtccggtgccctgaatgaactgcaggacgaggcagcgcggctatcgtggctggccacgacgggcgttccttgcgcagctgtgctcgacgttgtcactgaagcgggaagggactggctgctattgggcgaagtgccggggcaggatctcctgtcatctcaccttgctcctgccgagaaagtatccatcatggctgatgcaatgcggcggctgcatacgcttgatccggctacctgcccattcgaccaccaagcgaaacatcgcatcgagcgagcacgtactcggatggaagccggtcttgtcgatcaggatgatctggacgaagagcatcaggggctcgcgccagccgaactgttcgccaggctcaaggcgcgcatgcccgacggcgatgatctcgtcgtgacccatggcgatgcctgcttgccgaatatcatggtggaaaatggccgcttttctggattcatcgactgtggccggctgggtgtggcggaccgctatcaggacatagcgttggctacccgtgatattgctgaagagcttggcggcgaatgggctgaccgcttcctcgtgctttacggtatcgccgctcccgattcgcagcgcatcgccttctatcgccttcttgacgagttcttctgaggggatccgctgtaagtctgcagaaattgatgatctattaaacaataaagatgtccactaaaatggaagtttttcctgtcatactttgttaagaagggtgagaacagagtacctacattttgaatggaaggattggagctacgggggtgggggtggggtgggattagataaatgcctgctctttactgaaggctctttactattgctttatgataatgtttcatagttggatatcataatttaaacaagcaaaaccaaattaagggccagctcattcctcccactcatgatctatagatctatagatctctcgtgggatcattgtttttctcttgattcccactttgtggttctaagtactgtggtttccaaatgtgtcagtttcatagcctgaagaacgagatcagcagcctctgttccacatacacttcattctcagtattgttttgccaagttctaattccatcagacctcgacctgcagcccctagtcgagcgccagtagcagcacccacgtccaccttctgtctagtaatgtccaacacctccctcagtccaaacactgctctgcatccatgtggctcccatttatacctgaagcacttgatggggcctcaatgttttactagagcccacccccctgcaactctgagaccctctggatttgtctgtcagtgcctcactggggcgttggataatttcttaaaaggtcaagttccctcagcagcattctctgagcagtctgaagatgtgtgcttttcacagttcaaatccatgtggctgtttcacccacctgcctggccttgggttatctatcaggacctagcctagaagcaggtgtgtggcacttaacacctaagctgagtgactaactgaacactcaagtggatgccatctttgtcacttcttgactgtgacacaagcaactcctgatgccaaagccctgcccacccctctcatgcccatatttggacatggtacaggtcctcactggccatggtctgtgaggtcctggtcctctttgacttcataattcctaggggccactagtatctataagaggaagagggtgctggctcccaggccacagcccacaaaattccacctgctcacaggttggctggctcgacccaggtggtgtcccctgctctgagccagctcccggccaagccagcaccatgggaacccccaagaagaagaggaaggtgcgtaccgatttaaattccaatttactgaccgtacaccaaaatttgcctgcattaccggtcgatgcaacgagtgatgaggttcgcaagaacctgatggacatgttcagggatcgccaggcgttttctgagcatacctggaaaatgcttctgtccgtttgccggtcgtgggcggcatggtgcaagttgaataaccggaaatggtttcccgcagaacctgaagatgttcgcgattatcttctatatcttcaggcgcgcggtctggcagtaaaaactatccagcaacatttgggccagctaaacatgcttcatcgtcggtccgggctgccacgaccaagtgacagcaatgctgtttcactggttatgcggcggatccgaaaagaaaacgttgatgccggtgaacgtgcaaaacaggctctagcgttcgaacgcactgatttcgaccaggttcgttcactcatggaaaatagcgatcgctgccaggatatacgtaatctggcatttctggggattgcttataacaccctgttacgtatagccgaaattgccaggatcagggttaaagatatctcacgtactgacggtgggagaatgttaatccatattggcagaacgaaaacgctggttagcaccgcaggtgtagagaaggcacttagcctgggggtaactaaactggtcgagcgatggatttccgtctctggtgtagctgatgatccgaataactacctgttttgccgggtcagaaaaaatggtgttgccgcgccatctgccaccagccagctatcaactcgcgccctggaagggatttttgaagcaactcatcgattgatttacggcgctaaggtaaatataaaatttttaagtgtataatgtgttaaactactgattctaattgtttgtgtattttaggatgactctggtcagagatacctggcctggtctggacacagtgcccgtgtcggagccgcgcgagatatggcccgcgctggagtttcaataccggagatcatgcaagctggtggctggaccaatgtaaatattgtcatgaactatatccgtaacctggatagtgaaacaggggcaatggtgcgcctgctggaagatggcgattgatctagataagtaatgatcataatcagccatatcacatctgtagaggttttacttgctttaaaaaacctcccacacctccccctgaacctgaaacataaaatgaatgcaattgttgttgttaaacctgccctagttgcggccaattccagctgagcgtgagctcaccattaccagttggtctggtgtcaaaaataataataaccgggcaggggggatctaagctctagataagtaatgatcataatcagccatatcacatctgtagaggttttacttgctttaaaaaacctcccacacctccccctgaacctgaaacataaaatgaatgcaattgttgttgttaacttgtttattgcagcttataatggttacaaataaagcaatagcatcacaaatttcacaaataaagcatttttttcactgcattctagttgtggtttgtccaaactcatcaatgtatcttatcatgtctggatcctcgacataacttcgtataatgtatgctatacgaagttat

SEQ ID NO: 9 - DNA, 17210 bp, Artificial Sequence
  Polynucleotide sequence of a modified C9ORF72 locus from Exon 1a through 3' UTR
cgtttgtagtgacagccatcccaattgccctttccttctaggtggaaagtggtgtctagacagtccagggagggtgtgcgagggaggtgcgttttggttgcctcagctcgcaacttaactccacaacggtgaccaaggacaaaagaaggaaacaagactgcagagatccgcaccggggagccctgcagattctgggtctgctgtggactgggggcgggactgcgactgggcgggcctgggggcgtgtccggggcggggcggtcccggggcggggcccggagcgggctgcggttgcggtccctgcgccggcggtgaaggcgcagcagcggcgagtgggtgagtgagacgcgcgggcggaggggggctgctgccacggtcggctcgcgggccggccggctccgggtaccagcggggtttttttctccttcgaggtgaactcctccctgtcccccgggcgaaagagcccttggccttgcaggagttgcgggggccgcggcggtgcggaggggatggggatgggcctcatctttgctgtccgcccgcgctccccgatcccgacccggagcgtctcccgggcccttgagggaaccctccgggagtacggcgagcgcggcccccaccgccacaagcctgggccccaggggcctggcccggcgacagctggtgggtcctgcgacccagtcaggtctcccgagggtccccgcccgggaggagaaagcgccggtgggatggagtaaggacggacagaacaacacgcaggcaggatttcgcagaagtttgcaaggagtgcggatgcccacttacatgggctgctactcttaccaggttgttccccagttctgtgggacgtgacctggttgcctcacagctccgcggttgtacagacttattaaaggaagtgaccattgtgacttgggcatcacttgactgatggtaatcagttgcagagagagaagtgcactgattaagtctgtccacacagggtctgtctggccaggagtgcatttgcctgggagggattggttgcgctttctggtgtggggactattaggctcttgtagagttttgtcccggcagatggataaatttcttgttacactgttcccgttcgtcaccagttgagaaaaacgggtacacagtctgtctcagtagtacttttactttatattaagggcccaaaagggactggaaaatactttaagatagaatcgttagtccacttggaaaacttaaaatatgagagagagaggggggggggagagagagagagagagagagagagaaaggaaggaagaaggaggaagaggaggaggaaagagattgagattatgttaataatatggaatcagaatatttgaaatatagtaagcgtcccctcagttaaagaggacattccaggaggcccccagtatagcctgaaatctcaggaaacgcctacatacacccatcgtgtggatataggtgttttcccttcattacatttcatacacagatgttaaagtttagaaagtaggcacaataagagattacaaataactgataataaagtcgagccattgcagctgctctgtaaaagtcctgtgaatgtgatcgctttgtgtttcaaagtaacttactgtacttcacccctgttaagcaaaacaagattcacctgaacgcaggcaccttggtaccttggcagacaccagatctgataaccaagaggatggagaagtagtggcagacagtgtggagagcatgaatatgctagacaaaagggtgaatcataacctaggagcagaaagcaggtatttcatcatcctccacagtaaaaacctatgtcacgtaaaaaacctacaagtagtttttcttttactctttttgaatgaaagcttgctacaggcactgaaagttaaaataatctgtggatcaggaggaacaggggttttctgtctgagtcactgctgactagcacctcagtgaccattggcactgtgggaaaccccagagtcagttggaaacttcgaaactaaaggtgacggtgttcttatttcatagaacacaaaaaataagaggggttacagcctgcgctgcagactggacattcaacaagcatttaaatttctgggagacaaatgtaaatataactttaaaagttggtaaaatactctgtttggctatgttggccatccaatgtttgcttttagaaaatgactgaatggataaaacgtctatcttttgagcctgccctagacccccatgttgagtgaatactgtccaagtgttaggttagccggcctgagaaacttggatctaggcaagatggcacagtcctggtgtcatgagtatgcatgtgagttttggctgaaattgaacatttgtagagaatgacaaaggctggtctggcaagtagtccactgtctttacagtggtcttggttagttcctgtttggctgagagggctggttgatggctgtcctgcccctcttcccacaagtggaagccttatggtataattcttgatcacagtagcagtaggcaaatgaacttcctcaaagcagcctggaaagctgatttttttttctttctttctcttttttttttttttttcacaaggttaaagaaaaaacaaagggcttcaaatgtgccagtctgctaacagtgttaacatgtttattaacataaataaactttattagtttttggaagtattggttaagccctcgtgacccctgaactcggtttatagagtgatgagtcgtagcctcactctggtttggactctggcttctctcagaagactctgtggctaatgttaaccttctgaagtagccagaaaacatataagcaaaagtctgtgaggttgaaatgaattttttggccacatttgtatatgggttcccaccaatgctaacttcaggtgttagtaatatcagactcacagcttccctgattacacttcgctataagactttattttttaggtcataggaatttcccctttttcatgattcctaaatcatgaaataacatagtctaaaaatacggtattcctgaaataaacaatttctaagttttaagctgcgtgctattctgaacagtctgatgccctcttgtagcttttactgtgtcctaccccgggcatggttgattcctttgtccaaacatctgtctgttgtatccacactggattgcaccacctgcgtgctagtcagtcactcagacattttagttataaggtagcttatatttactccttattttatttaataatggcctcatagcaaggcggtaatgatactggtaatttgggtttgcttaagaggagccatgaagtagttttaaatgaaaaggtgaaaattcccactatagtttggagggggaggctatactggtactactacgattcacggtaagactaaatcttctgtgaaattatgaaggagaaaaagttacactggtctggtcttgctgttggattaattttatagttataaccactgtacatgataaataaccctaaaacaatgaatttgtaggtggatggcataatctgaaaaccatgttctgagcagttgatggcagcaggctgtgctggaagtgttaggcatatttatagatttcagcccaagttctgaagaggctggagagatggctcagtggttaagagtgcttgctattgcagaggacctaggttcctctacaggcaccaggcaagcgtgggacacactgagatacatacagacaaaacataaaattaaataaattgtgcataataatactagtaatatatgagtaaaataaggataaatacacatcataattaaataaataaattgtaaagttccctagaagtgagggtcaccaagccattcacaagatggctgcgctgatgcagggatatatgtgaactagaaaaaggtcaaacttaacagagaagttccaaggcatgctactgcaggcttggctagcatgcttgacctgcagaaatgctgacggccactgggaggttttcacaaatgaggaattagaagaactttttttactaatctccagaaaaaaaaaagggaagaagaaactgaagcagcctgtgatgtggaccagaaacgcagtgacagtaacatgtgtgacattgcaaaggcatgaaaggacagagctgtggaatacagacctcaggtggagctcagcatagagtcattcggggattatgcctgctgcagcaacaaaaggatgagctcaaaagagacaccgacttctgaatgcagtgggtgtttgttttgttttgtttcaaatgaattgggcagaaaactttccagctgtggaagcttctgaaccgtcccttgctgctgacatctaagcgtccgctgtgtcccagctcagtgatctagggtcttccaaacagatggtccggtgctgagcactttgaatctcaatcctgagtttctaccacgcctttggccatttaattcccagataaaagacacatacaacctttatatttataataaaccttagtcagcacaagagctgagcaaatatctgtcctctatgctattatatctattacccagccaataaccccattctataatttgctgtgcttcatctgggctgctcttaacttcagtcagccagcccacgtggccattattttaagatttttttaccccatagtgtcttctcactttactttacatttttctctctctcctcatggttctcctctgaccccaagcctaggaaccctaaaccccacccatgtctcttctgcccatctattggctgtaggcatctttattcaccaatcaggataacttggaggcaaggttaagtagtctcctgggtctaggtgctgtctctgggagcaaccagtatttagcatagcaaaagaccagacctccacaatgatcactctgaccatcggggcagaaggcacctactagcctgtgccactcacctcactttgttgaatcacatcttatcctgtagtgtgtatcactgcctgttatcacaggaaaaagtgagtcccatcaaataagatgtttcagaaagagaccatgttcatataattatcattctggtaagcttttaatggttatattttgttattaatctctttgttcctattttgcaaattataccttacagtaaatatatatgcatccaatggggtctttgaattcctccccggggagtaggaggactctttgaggatgggctgcatttaaagctaaacaacgcaacatgacctttagtccttatagatagcctagagatgagactaaataaaagaaatggtatataatgctttaagtttcccaatcagcttaaaagcttttcctataaatctttaagattatgctctggggctcaatactgcttcaagaagggcttttcttttgtatttagaattattcacctttttaaacaaaaggagaaaatggaatagaaatatgtttgcaacataattttatgactatgtgtttatttcgcgtgttctgtgggcctgcagtttgctgctgttaatgaggacaacagtggcaccaatacagtttccactcagattacattctctgttccctttctgaaagctgccctctccactgggcccaaaagagtcagtatcttaaacaagctgtacaacttagataaccatggtctcttcagactagttaattgacatatattaaaaagtaaatagtaccaaagtgaatttctgaaattaaaaatgaacatttaaaaactctaggtaaactattccttagagttaagtgttttgccaagttctgtaatcataatatgatagaaacgctcactcagcattctaaatatagaagttactccttcgcatgacactctaattcttgataaggtggagaaagagagagagagagggggagagacagaaaatatggtggttcaaggaccatttgagggaattagttatgttcttccgtcctctgtggatcttaggggttgaatacagtcattgagctcggtggatggctgtcctgttgaaaggtctgcccagcagagcaaatagacttttttatttacatggacatccgtttgtgactaatctaatgttcactcccaaagtaatcacacagacagagaggtagcttccttcagtactcttaccttacatgaatcctaccattttgttattttttttccactttaaatctttgattatgtgtttttaattagaaaatttgcatacaaatttccatacagtatgtagaattgactgtgtttgaatgggtgaagatccacatgtgtaaccctagctctggactggctctgagcttgtttgctcttctcttttgtgttctgagtaactgaaactctttcattttagcagcttagtatgcgcccttcacattgctgtgctgcctgctgcactaacattactcctttgcttatgttccccttcctgattcagtgtcattttaagcagtagtactggacctcagtaccttagccggagctcactgaggtgacagggctgaggctctgctgctgtcttttgagcttacctctttttaatgttttatggtatttctgctgccaggtttgggggttttgttttgttttgttttttgttttttgttttttttaattttctaggaacacctagaaaacacaaactaggaaacttaaaagagcagcgtcttgttccctgcgttctagaaagtccaagcctaatgccagtgtcatggttgtcaggaacatgagcctctgaaggcttcttgggaaacctttcttgtctcaacacctctggtggcaagcagtagtccatggtactctctctgtccacggtcagcatcccagtccctgccctttatctttgtgcagccgaccagctttgctttagtctgtctccttctcaggtctccttccccgctcctcttaagcacagcagtcattggattagagcccatccttccctcggatggcccatttgacctaattttacgtatttgtaactaaggtcccatttacttacacagggccctccccttcctgttttgttctttagctgaaatggtttggagaccaaatatccaatcattacaattgtgcacaagctatgttcatttggaggtaataaaggctcattctttgcttctattggtatgtgacatttttctaagtcacttggggtttgatagatatctttaaatggctgaacctgatcactgttcttttgtatgtccctgtttagctattgcaagcgttcggataatgtgagacctggaatgcagtgagacctgggatgcagggatgggtaccgatttaaatgatccagtggtcctgcagaggagagattgggagaatcccggtgtgacacagctgaacagactagccgcccaccctccctttgcttcttggagaaacagtgaggaagctaggacagacagaccaagccagcaactcagatctttgaacggggagtggagatttgcctggtttccggcaccagaagcggtgccggaaagctggctggagtgcgatcttcctgaggccgatactgtcgtcgtcccctcaaactggcagatgcacggttacgatgcgcccatctacaccaacgtgacctatcccattacggtcaatccgccgtttgttcccacggagaatccgacgggttgttactcgctcacatttaatgttgatgaaagctggctacaggaaggccagacgcgaattatttttgatggcgttaactcggcgtttcatctgtggtgcaacgggcgctgggtcggttacggccaggacagtcgtttgccgtctgaatttgacctgagcgcatttttacgcgccggagaaaaccgcctcgcggtgatggtgctgcgctggagtgacggcagttatctggaagatcaggatatgtggcggatgagcggcattttccgtgacgtctcgttgctgcataaaccgactacacaaatcagcgatttccatgttgccactcgctttaatgatgatttcagccgcgctgtactggaggctgaagttcagatgtgcggcgagttgcgtgactacctacgggtaacagtttctttatggcagggtgaaacgcaggtcgccagcggcaccgcgcctttcggcggtgaaattatcgatgagcgtggtggttatgccgatcgcgtcacactacgtctgaacgtcgaaaacccgaaactgtggagcgccgaaatcccgaatctctatcgtgcggtggttgaactgcacaccgccgacggcacgctgattgaagcagaagcctgcgatgtcggtttccgcgaggtgcggattgaaaatggtctgctgctgctgaacggcaagccgttgctgattcgaggcgttaaccgtcacgagcatcatcctctgcatggtcaggtcatggatgagcagacgatggtgcaggatatcctgctgatgaagcagaacaactttaacgccgtgcgctgttcgcattatccgaaccatccgctgtggtacacgctgtgcgaccgctacggcctgtatgtggtggatgaagccaatattgaaacccacggcatggtgccaatgaatcgtctgaccgatgatccgcgctggctaccggcgatgagcgaacgcgtaacgcgaatggtgcagcgcgatcgtaatcacccgagtgtgatcatctggtcgctggggaatgaatcaggccacggcgctaatcacgacgcgctgtatcgctggatcaaatctgtcgatccttcccgcccggtgcagtatgaaggcggcggagccgacaccacggccaccgatattatttgcccgatgtacgcgcgcgtggatgaagaccagcccttcccggctgtgccgaaatggtccatcaaaaaatggctttcgctacctggagagacgcgcccgctgatcctttgcgaatacgcccacgcgatgggtaacagtcttggcggtttcgctaaatactggcaggcgtttcgtcagtatccccgtttacagggcggcttcgtctgggactgggtggatcagtcgctgattaaatatgatgaaaacggcaacccgtggtcggcttacggcggtgattttggcgatacgccgaacgatcgccagttctgtatgaacggtctggtctttgccgaccgcacgccgcatccagcgctgacggaagcaaaacaccagcagcagtttttccagttccgtttatccgggcaaaccatcgaagtgaccagcgaatacctgttccgtcatagcgataacgagctcctgcactggatggtggcgctggatggtaagccgctggcaagcggtgaagtgcctctggatgtcgctccacaaggtaaacagttgattgaactgcctgaactaccgcagccggagagcgccgggcaactctggctcacagtacgcgtagtgcaaccgaacgcgaccgcatggtcagaagccgggcacatcagcgcctggcagcagtggcgtctggcggaaaacctcagtgtgacgctccccgccgcgtcccacgccatcccgcatctgaccaccagcgaaatggatttttgcatcgagctgggtaataagcgttggcaatttaaccgccagtcaggctttctttcacagatgtggattggcgataaaaaacaactgctgacgccgctgcgcgatcagttcacccgtgcaccgctggataacgacattggcgtaagtgaagcgacccgcattgaccctaacgcctgggtcgaacgctggaaggcggcgggccattaccaggccgaagcagcgttgttgcagtgcacggcagatacacttgctgatgcggtgctgattacgaccgctcacgcgtggcagcatcaggggaaaaccttatttatcagccggaaaacctaccggattgatggtagtggtcaaatggcgattaccgttgatgttgaagtggcgagcgatacaccgcatccggcgcggattggcctgaactgccagctggcgcaggtagcagagcgggtaaactggctcggattagggccgcaagaaaactatcccgaccgccttactgccgcctgttttgaccgctgggatctgccattgtcagacatgtataccccgtacgtcttcccgagcgaaaacggtctgcgctgcgggacgcgcgaattgaattatggcccacaccagtggcgcggcgacttccagttcaacatcagccgctacagtcaacagcaactgatggaaaccagccatcgccatctgctgcacgcggaagaaggcacatggctgaatatcgacggtttccatatggggattggtggcgacgactcctggagcccgtcagtatcggcggaattccagctgagcgccggtcgctaccattaccagttggtctggtgtcaaaaataataataaccgggcaggggggatctaagctctagataagtaatgatcataatcagccatatcacatctgtagaggttttacttgctttaaaaaacctcccacacctccccctgaacctgaaacataaaatgaatgcaattgttgttgttaacttgtttattgcagcttataatggttacaaataaagcaatagcatcacaaatttcacaaataaagcatttttttcactgcattctagttgtggtttgtccaaactcatcaatgtatcttatcatgtctggatcccccggctagagtttaaacactagaactagtggatccccgggctcgataactataacggtcctaaggtagcgactcgagataacttcgtataatgtatgctatacgaagttatatgcatggcctccgcgccgggttttggcgcctcccgcgggcgcccccctcctcacggcgagcgctgccacgtcagacgaagggcgcagcgagcgtcctgatccttccgcccggacgctcaggacagcggcccgctgctcataagactcggccttagaaccccagtatcagcagaaggacattttaggacgggacttgggtgactctagggcactggttttctttccagagagcggaacaggcgaggaaaagtagtcccttctcggcgattctgcggagggatctccgtggggcggtgaacgccgatgattatataaggacgcgccgggtgtggcacagctagttccgtcgcagccgggatttgggtcgcggttcttgtttgtggatcgctgtgatcgtcacttggtgagtagcgggctgctgggctggccggggctttcgtggccgccgggccgctcggtgggacggaagcgtgtggagagaccgccaagggctgtagtctgggtccgcgagcaaggttgccctgaactgggggttggggggagcgcagcaaaatggcggctgttcccgagtcttgaatggaagacgcttgtgaggcgggctgtgaggtcgttgaaacaaggtggggggcatggtgggcggcaagaacccaaggtcttgaggccttcgctaatgcgggaaagctcttattcgggtgagatgggctggggcaccatctggggaccctgacgtgaagtttgtcactgactggagaactcggtttgtcgtctgttgcgggggcggcagttatggcggtgccgttgggcagtgcacccgtacctttgggagcgcgcgccctcgtcgtgtcgtgacgtcacccgttctgttggcttataatgcagggtggggccacctgccggtaggtgtgcggtaggcttttctccgtcgcaggacgcagggttcgggcctagggtaggctctcctgaatcgacaggcgccggacctctggtgaggggagggataagtgaggcgtcagtttctttggtcggttttatgtacctatcttcttaagtagctgaagctccggttttgaactatgcgctcggggttggcgagtgtgttttgtgaagttttttaggcaccttttgaaatgtaatcatttgggtcaatatgtaattttcagtgttagactagtaaattgtccgctaaattctggccgtttttggcttttttgttagacgtgttgacaattaatcatcggcatagtatatcggcatagtataatacgacaaggtgaggaactaaaccatgggatcggccattgaacaagatggattgcacgcaggttctccggccgcttgggtggagaggctattcggctatgactgggcacaacagacaatcggctgctctgatgccgccgtgttccggctgtcagcgcaggggcgcccggttctttttgtcaagaccgacctgtccggtgccctgaatgaactgcaggacgaggcagcgcggctatcgtggctggccacgacgggcgttccttgcgcagctgtgctcgacgttgtcactgaagcgggaagggactggctgctattgggcgaagtgccggggcaggatctcctgtcatctcaccttgctcctgccgagaaagtatccatcatggctgatgcaatgcggcggctgcatacgcttgatccggctacctgcccattcgaccaccaagcgaaacatcgcatcgagcgagcacgtactcggatggaagccggtcttgtcgatcaggatgatctggacgaagagcatcaggggctcgcgccagccgaactgttcgccaggctcaaggcgcgcatgcccgacggcgatgatctcgtcgtgacccatggcgatgcctgcttgccgaatatcatggtggaaaatggccgcttttctggattcatcgactgtggccggctgggtgtggcggaccgctatcaggacatagcgttggctacccgtgatattgctgaagagcttggcggcgaatgggctgaccgcttcctcgtgctttacggtatcgccgctcccgattcgcagcgcatcgccttctatcgccttcttgacgagttcttctgaggggatccgctgtaagtctgcagaaattgatgatctattaaacaataaagatgtccactaaaatggaagtttttcctgtcatactttgttaagaagggtgagaacagagtacctacattttgaatggaaggattggagctacgggggtgggggtggggtgggattagataaatgcctgctctttactgaaggctctttactattgctttatgataatgtttcatagttggatatcataatttaaacaagcaaaaccaaattaagggccagctcattcctcccactcatgatctatagatctatagatctctcgtgggatcattgtttttctcttgattcccactttgtggttctaagtactgtggtttccaaatgtgtcagtttcatagcctgaagaacgagatcagcagcctctgttccacatacacttcattctcagtattgttttgccaagttctaattccatcagacctcgacctgcagcccctagtcgagcgccagtagcagcacccacgtccaccttctgtctagtaatgtccaacacctccctcagtccaaacactgctctgcatccatgtggctcccatttatacctgaagcacttgatggggcctcaatgttttactagagcccacccccctgcaactctgagaccctctggatttgtctgtcagtgcctcactggggcgttggataatttcttaaaaggtcaagttccctcagcagcattctctgagcagtctgaagatgtgtgcttttcacagttcaaatccatgtggctgtttcacccacctgcctggccttgggttatctatcaggacctagcctagaagcaggtgtgtggcacttaacacctaagctgagtgactaactgaacactcaagtggatgccatctttgtcacttcttgactgtgacacaagcaactcctgatgccaaagccctgcccacccctctcatgcccatatttggacatggtacaggtcctcactggccatggtctgtgaggtcctggtcctctttgacttcataattcctaggggccactagtatctataagaggaagagggtgctggctcccaggccacagcccacaaaattccacctgctcacaggttggctggctcgacccaggtggtgtcccctgctctgagccagctcccggccaagccagcaccatgggaacccccaagaagaagaggaaggtgcgtaccgatttaaattccaatttactgaccgtacaccaaaatttgcctgcattaccggtcgatgcaacgagtgatgaggttcgcaagaacctgatggacatgttcagggatcgccaggcgttttctgagcatacctggaaaatgcttctgtccgtttgccggtcgtgggcggcatggtgcaagttgaataaccggaaatggtttcccgcagaacctgaagatgttcgcgattatcttctatatcttcaggcgcgcggtctggcagtaaaaactatccagcaacatttgggccagctaaacatgcttcatcgtcggtccgggctgccacgaccaagtgacagcaatgctgtttcactggttatgcggcggatccgaaaagaaaacgttgatgccggtgaacgtgcaaaacaggctctagcgttcgaacgcactgatttcgaccaggttcgttcactcatggaaaatagcgatcgctgccaggatatacgtaatctggcatttctggggattgcttataacaccctgttacgtatagccgaaattgccaggatcagggttaaagatatctcacgtactgacggtgggagaatgttaatccatattggcagaacgaaaacgctggttagcaccgcaggtgtagagaaggcacttagcctgggggtaactaaactggtcgagcgatggatttccgtctctggtgtagctgatgatccgaataactacctgttttgccgggtcagaaaaaatggtgttgccgcgccatctgccaccagccagctatcaactcgcgccctggaagggatttttgaagcaactcatcgattgatttacggcgctaaggtaaatataaaatttttaagtgtataatgtgttaaactactgattctaattgtttgtgtattttaggatgactctggtcagagatacctggcctggtctggacacagtgcccgtgtcggagccgcgcgagatatggcccgcgctggagtttcaataccggagatcatgcaagctggtggctggaccaatgtaaatattgtcatgaactatatccgtaacctggatagtgaaacaggggcaatggtgcgcctgctggaagatggcgattgatctagataagtaatgatcataatcagccatatcacatctgtagaggttttacttgctttaaaaaacctcccacacctccccctgaacctgaaacataaaatgaatgcaattgttgttgttaaacctgccctagttgcggccaattccagctgagcgtgagctcaccattaccagttggtctggtgtcaaaaataataataaccgggcaggggggatctaagctctagataagtaatgatcataatcagccatatcacatctgtagaggttttacttgctttaaaaaacctcccacacctccccctgaacctgaaacataaaatgaatgcaattgttgttgttaacttgtttattgcagcttataatggttacaaataaagcaatagcatcacaaatttcacaaataaagcatttttttcactgcattctagttgtggtttgtccaaactcatcaatgtatcttatcatgtctggatcctcgacataacttcgtataatgtatgctatacgaagttattgctagcgtgtctcagcagtgtgtgggcacatccttcctcccgagtcctgctgcaggacagggtacactacacttgtcagtagaagtctgtacctgatgtcaggtgcatcgttacagtgaatgactcttcctagaatagatgtactcttttagggccttatgtttacaattatcctaagtactattgctgtcttttaaagatatgaatgatggaatatacacttgaccataactgctgattggttttttgttttgttttgtttgttttcttggaaacttatgattcctggtttacatgtaccacactgaaaccctcgttagctttacagataaagtgtgagttgacttcctgcccctctgtgttctgtggtatgtccgattacttctgccacagctaaacattagagcatttaaagtttgcagttcctcagaaaggaacttagtctgactacagattagttcttgagagaagacactgatagggcagagctgtaggtgaaatcagttgttagcccttcctttatagacgtagtccttcagattcggtctgtacagaaatgccgaggggtcatgcatgggccctgagtatcgtgacctgtgacaagttttttgttggtttattgtagttctgtcaaagaaagtggcatttgtttttataattgttgccaacttttaaggttaattttcattatttttgagccgaattaaaatgcgcacctcctgtgcctttcccaatcttggaaaatataatttcttggcagagggtcagatttcagggcccagtcactttcatctgaccaccctttgcacggctgccgtgtgcctggcttagattagaagtccttgttaagtatgtcagagtacattcgctgataagatctttgaagagcagggaagcgtcttgcctctttcctttggtttctgcctgtactctggtgtttcccgtgtcacctgcatcataggaacagcagagaaatctgacccagtgctatttttctaggtgctactatggcaaactcaagtggtctgtttctgttcctgtaacgttcgactatctcgctagctgtgaagtactgattagtggagttctgtgcaacagcagtgtaggagtatacacaaacacaaatatgtgtttctatttaaaactgtggacttagcataaaaagggagaatatatttattttttacaaaagggataaaaatgggccccgttcctcacccaccagatttagcgagaaaaagctttctattctgaaaggtcacggtggctttggcattacaaatcagaacaacacacactgaccatgatggcttgtgaactaactgcaaggcactccgtcatggtaagcgagtaggtcccacctcctagtgtgccgctcattgctttacacagtagaatcttatttgagtgctaattgttgtctttgctgctttactgtgttgttatagaaaatgtaagctgtacagtgaataagttattgaagcatgtgtaaacactgttatatatcttttctcctagatggggaattttgaataaaatacctttgaaattc